European Patent Specification EP 3 769 784 B1, published September 13, 2023. Title: Composition for suppressing inflammation. Applicant: Kyoto University. The sequence listing filed with the application follows.

SEQUENCE LISTING (14 sequences)

SEQ ID NO: 1 - RNA, 765 nt, Homo sapiens
gcugccuguggcuggcaagggcagcacccccagccuccaagggccgucaggcugggcuuugggccauugagcagcccauucccagcccugaggcccaccccagaggcuggacagagggaggauucaagucgggaaggaaacccacaaaccaaagauacuguaggauugguucuggcccaugcagcaccucuagcugucugccucagugggucagaagcgaucacccuguugauacacauuguaucucuguaguuuaaggagacgcugccgguaacggcgucgguccguggcugaggcccaaaccgucuuuucucucagaggguggggagggaggugggggcagcagaggccugggcugggugcccugugcacgccaccccacuuccgcccuaccccugggacguuggccuuggcuggcuaguugggcaccgugugccugcccuccaagggccuccucuacgccaaugaggccucaucugugcucucgcugggcacguggcuucaugucaguaagcaagaugcuucuuaauaacccaccuucugccccacucuauuccuuauccugcugccccuguaggggucaagggcccuccgucuacacccucuucuucuccuccauccuuuauucagagucaucucgcccuuccccaugggugggggaaccuguguuuguuugugugcacauguaaauuuuaaauauuuuaagcagaaaguccuuaccuccuguaacacaucaauaaaguacaaucauugugagcccuuuca

SEQ ID NO: 2 - RNA, 865 nt, Mus musculus
gccagaagguggcgcaaggggcugucgggcaucacagauagcgguccccagccccugccuggccuacccuggaagcuggacagaaggacaagugaagcaggcaagggaauccucaaaccaaagauaccauaggauugguucuggccccgcggcaccccaacccgucccgcacaggucagaagugaucacccuguugauacacauuguaucucugucauuuaaggagacgcugccggucaggccguccauccguggcugaugcccaaacccucuuuuuuuuuucucagagggccgggugggaggcaugggggagcagaggccugagcuggaccccaccuuccacccugucccugggacgccggcaccaccggcuaguuaggcaccaugugccugcucucugaggcccccucaagccaaugcggccucaucccuguucacagggcaugaggcuucauguuaguaagcaagaugcuucuuuaagccccuccccugcccgcucuguccaccuacacaccccccccccaaccagggcuccaaggcccucuguuuccacaccucccaugggugggaggacacauguaugcuguguacagaggcgagauuuaaauauuuuaaaugaaaaagguugacaaaauaaaggcuauugccaggcaggcuggagagauggcucagugguuaagagcaccgacugcucuucugaagguccugaguucaaaugucagcaaccacaugguggcucacaaacaucugugaugagaucuggugcccucuucuggggugucugaagacagcuacaguguacuuacauacaauaauaaaucuuuuaaaaaagagagaaauuuaaaagaaaaaaaaagcuauugcc

SEQ ID NO: 3 - protein, 599 aa, Homo sapiens
MSGPCGEKPVLEASPTMSLWEFEDSHSRQGTPRPGQELAAEEASALELQMKVDFFRKLGYSSTEIHSVLQKLGVQADTNTVLGELVKHGTATERERQTSPDPCPQLPLVPRGGGTPKAPNLEPPLPEEEKEGSDLRPVVIDGSNVAMSHGNKEVFSCRGILLAVNWFLERGHTDITVFVPSWRKEQPRPDVPITDQHILRELEKKKILVFTPSRRVGGKRVVCYDDRFIVKLAYESDGIVVSNDTYRDLQGERQEWKRFIEERLLMYSFVNDKFMPPDDPLGRHGPSLDNFLRKKPLTLEHRKQPCPYGRKCTYGIKCRFFHPERPSCPQRSVADELRANALLSPPRAPSKDKNGRRPSPSSQSSSLLTESEQCSLDGKKLGAQASPGSRQEGLTQTYAPSGRSLAPSGGSGSSFGPTDWLPQTLDSLPYVSQDCLDSGIGSLESQMSELWGVRGGGPGEPGPPRAPYTGYSPYGSELPATAAFSAFGRAMGAGHFSVPADYPPAPPAFPPREYWSEPYPLPPPTSVLQEPPVQSPGAGRSPWGRAGSLAKEQASVYTKLCGVFPPHLVEAVMGRFPQLLDPQQLAAEILSYKSQHPSE

SEQ ID NO: 4 - protein, 596 aa, Mus musculus
MSDPCGTKPVQESNPTMSLWSLEDRHSSQGRPQPDQDPVAKEAPTSELQMKVDFFRKLGYSSSEIHSVLQKLGVQADTNTVLGELVKHGSATERECQALTAPSPQPPLVPRGGSTPKPSTLEPSLPEEDREGSDLRPVVIDGSNVAMSHGNKEVFSCRGILLAVNWFLERGHTDITVFVPSWRKEQPRPDVPITDQHILRELEKKKILVFTPSRRVGGKRVVCYDDRFIVKLAFESDGVVVSNDTYRDLQGERQEWKRFIEERLLMYSFVNDKFMPPDDPLGRHGPSLDNFLRKKPLPSEHRKQPCPYGKKCTYGIKCRFFHPERPSRPQRSVADELRANALLSPPRTPVKDKSSQRPSPASQSSSVSLEAEPGSLDGKKLGARSSPGPHREGSPQTCAPAGRSLPVSGGSFGPTEWLAHTQDSLPYTSQECLDSGIGSLESQMSELWGVRGGSPGESGPTRGPYAGYHSYGSKVPAAPSFSPFRPAMGAGHFSVPTDYVPPPPTYPSREYWSEPYPLPPPTPVLQEPQRPSPGAGGGPWGRVGDLAKERAGVYTKLCGVFPPHLVEAVMRRFPQLLDPQQLAAEILSYKSQHLSE

SEQ ID NO: 5 - RNA, 262 nt, Homo sapiens
gugggucagaagcgaucacccuguugauacacauuguaucucuguaguuuaaggagacgcugccgguaacggcgucgguccguggcugaggcccaaaccgucuuuucucucagaggguggggagggaggugggggcagcagaggccugggcugggugcccugugcacgccaccccacuuccgcccuaccccugggacguuggccuuggcuggcuaguugggcaccgugugccugcccuccaagggccuccucuacgccaaug

SEQ ID NO: 6 - RNA, 246 nt, Mus musculus
acaggucagaagugaucacccuguugauacacauuguaucucugucauuuaaggagacgcugccggucaggccguccauccguggcugaugcccaaacccucuuuuuuuuuucucagagggccgggugggaggcaugggggagcagaggccugagcuggaccccaccuuccacccugucccugggacgccggcaccaccggcuaguuaggcaccaugugccugcucucugaggcccccucaagcca

SEQ ID NO: 7 - DNA, 23 bp, Homo sapiens
aatgtgtatcaacagggtgatcg

SEQ ID NO: 8 - DNA, 23 bp, Homo sapiens
cttaaactacagagatacaatgt

SEQ ID NO: 9 - DNA, 19 bp, Homo sapiens
acggtgcccaactagccag

SEQ ID NO: 10 - DNA, 19 bp, Homo sapiens
ggcccttggagggcaggca

SEQ ID NO: 11 - DNA, 23 bp, Mus musculus
aatgtgtatcaacagggtgatca

SEQ ID NO: 12 - DNA, 23 bp, Mus musculus
cttaaatgacagagatacaatgt

SEQ ID NO: 13 - DNA, 20 bp, Mus musculus
atggtgcctaactagccggt

SEQ ID NO: 14 - DNA, 20 bp, Mus musculus
cctcagagagcaggcacatg